European Patent Specification EP 3 630 961 B1, published June 26, 2024. Title: Genetic Construct. Applicant: MacDonald, Mike. The sequence listing filed with the application follows.

SEQUENCE LISTING (31 sequences)

SEQ ID NO: 1 - DNA, 1494 bp, Homo sapiens
atgcccacccccgacgccaccacgccacaggccaagggcttccgcagggccgtgtctgagctggacgccaagcaggcagaggccatcatgtccccgcggttcattgggcgcaggcagagcctcatcgaggacgcccgcaaggagcgggaggcggcggtggcagcagcggccgctgcagtcccctcggagcccggggaccccctggaggctgtggcctttgaggagaaggaggggaaggccgtgctaaacctgctcttctccccgagggccaccaagccctcggcgctgtcccgagctgtgaaggtgtttgagacgtttgaagccaaaatccaccatctagagacccggcccgcccagaggccgcgagctgggggcccccacctggagtacttcgtgcgcctcgaggtgcgccgaggggacctggccgccctgctcagtggtgtgcgccaggtgtcagaggacgtgcgcagccccgcggggcccaaggtcccctggttcccaagaaaagtgtcagagctggacaagtgtcatcacctggtcaccaagttcgaccctgacctggacttggaccacccgggcttctcggaccaggtgtaccgccagcgcaggaagctgattgctgagatcgccttccagtacaggcacggcgacccgattccccgtgtggagtacaccgccgaggagattgccacctggaaggaggtctacaccacgctgaagggcctctacgccacgcacgcctgcggggagcacctggaggcctttgctttgctggagcgcttcagcggctaccgggaagacaatatcccccagctggaggacgtctcccgcttcctgaaggagcgcacgggcttccagctgcggcctgtggccggcctgctgtccgcccgggacttcctggccagcctggccttccgcgtgttccagtgcacccagtatatccgccacgcgtcctcgcccatgcactcccctgagccggactgctgccacgagctgctggggcacgtgcccatgctggccgaccgcaccttcgcgcagttctcgcaggacattggcctggcgtccctgggggcctcggatgaggaaattgagaagctgtccacgctgtactggttcacggtggagttcgggctgtgtaagcagaacggggaggtgaaggcctatggtgccgggctgctgtcctcctacggggagctcctgcactgcctgtctgaggagcctgagattcgggccttcgaccctgaggctgcggccgtgcagccctaccaagaccagacgtaccagtcagtctacttcgtgtctgagagcttcagtgacgccaaggacaagctcaggagctatgcctcacgcatccagcgccccttctccgtgaagttcgacccgtacacgctggccatcgacgtgctggacagcccccaggccgtgcggcgctccctggagggtgtccaggatgagctggacacccttgcccatgcgctgagtgccattggctag

SEQ ID NO: 2 - DNA, 1029 bp, Homo sapiens
atgagccccgcggggcccaaggtcccctggttcccaagaaaagtgtcagagctggacaagtgtcatcacctggtcaccaagttcgaccctgacctggacttggaccacccgggcttctcggaccaggtgtaccgccagcgcaggaagctgattgctgagatcgccttccagtacaggcacggcgacccgattccccgtgtggagtacaccgccgaggagattgccacctggaaggaggtctacaccacgctgaagggcctctacgccacgcacgcctgcggggagcacctggaggcctttgctttgctggagcgcttcagcggctaccgggaagacaatatcccccagctggaggacgtctcccgcttcctgaaggagcgcacgggcttccagctgcggcctgtggccggcctgctgtccgcccgggacttcctggccagcctggccttccgcgtgttccagtgcacccagtatatccgccacgcgtcctcgcccatgcactcccctgagccggactgctgccacgagctgctggggcacgtgcccatgctggccgaccgcaccttcgcgcagttctcgcaggacattggcctggcgtccctgggggcctcggatgaggaaattgagaagctgtccacgctgtactggttcacggtggagttcgggctgtgtaagcagaacggggaggtgaaggcctatggtgccgggctgctgtcctcctacggggagctcctgcactgcctgtctgaggagcctgagattcgggccttcgaccctgaggctgcggccgtgcagccctaccaagaccagacgtaccagtcagtctacttcgtgtctgagagcttcagtgacgccaaggacaagctcaggagctatgcctcacgcatccagcgccccttctccgtgaagttcgacccgtacacgctggccatcgacgtgctggacagcccccaggccgtgcggcgctccctggagggtgtccaggatgagctggacacccttgcccatgcgctgagtgccattggctag

SEQ ID NO: 3 - DNA, 792 bp, Mus musculus
ggtggttttcctttgaaaaacacgatgataatatggccacaaccgcggccgtagatcccgggaccatggagaagccgcggggagtcaggtgcaccaatgggttctccgagcgggagctgccgcggcccggggccagcccgcctgccgagaagtcccggccgcccgaggccaagggcgcacagccggccgacgcctggaaggcagggcggcaccgcagcgaggaggaaaaccaggtgaacctccccaaactggcggctgcttactcgtccattctgctctcgctgggcgaggacccccagcggcaggggctgctcaagacgccctggagggcggccaccgccatgcagtacttcaccaagggataccaggagaccatctcagatgtcctgaatgatgctatatttgatgaagatcatgacgagatggtgattgtgaaggacatagatatgttctccatgtgtgagcatcaccttgttccatttgtaggaagggtccatattggctatcttcctaacaagcaagtccttggtctcagtaaacttgccaggattgtagaaatctacagtagacgactacaagttcaagagcgcctcaccaaacagattgcggtggccatcacagaagccttgcagcctgctggcgttggagtagtgattgaagcgacacacatgtgcatggtaatgcgaggcgtgcagaaaatgaacagcaagactgtcactagcaccatgctgggcgtgttccgggaagaccccaagactcgggaggagttcctcacactaatcaggagctgag

SEQ ID NO: 4 - DNA, 753 bp, Homo sapiens
atggagaagggccctgtgcgggcaccggcggagaagccgcggggcgccaggtgcagcaatgggttccccgagcgggatccgccgcggcccgggcccagcaggccggcggagaagcccccgcggcccgaggccaagagcgcgcagcccgcggacggctggaagggcgagcggccccgcagcgaggaggataacgagctgaacctccctaacctggcagccgcctactcgtccatcctgagctcgctgggcgagaacccccagcggcaagggctgctcaagacgccctggagggcggcctcggccatgcagttcttcaccaagggctaccaggagaccatctcagatgtcctaaacgatgctatatttgatgaagatcatgatgagatggtgattgtgaaggacatagacatgttttccatgtgtgagcatcacttggttccatttgttggaaaggtccatattggttatcttcctaacaagcaagtccttggcctcagcaaacttgcgaggattgtagaaatctatagtagaagactacaagttcaggagcgccttacaaaacaaattgctgtagcaatcacggaagccttgcggcctgctggagtcggggtagtggttgaagcaacacacatgtgtatggtaatgcgaggtgtacagaaaatgaacagcaaaactgtgaccagcacaatgttgggtgtgttccgggaggatccaaagactcgggaagagttcctgactctcattaggagctga

SEQ ID NO: 5 - DNA, 469 bp, Homo sapiens
ctgcagagggccctgcgtatgagtgcaagtgggttttaggaccaggatgaggcggggtgggggtgcctacctgacgaccgaccccgacccactggacaagcacccaacccccattccccaaattgcgcatcccctatcagagagggggaggggaaacaggatgcggcgaggcgcgtgcgcactgccagcttcagcaccgcggacagtgccttcgcccccgcctggcggcgcgcgccaccgccgcctcagcactgaaggcgcgctgacgtcactcgccggtcccccgcaaactccccttcccggccaccttggtcgcgtccgcgccgccgccggcccagccggaccgcaccacgcgaggcgcgagataggggggcacgggcgcgaccatctgcgctgcggcgccggcgactcagcgctgcctcagtctgcggtgggcagcggaggagtcgtgtcgtgcctgagagcgcag

SEQ ID NO: 6 - DNA, 461 bp, Foot-and-mouth disease virus
agcaggtttccccaactgacacaaaacgtgcaacttgaaactccgcctggtctttccaggtctagaggggtaacactttgtactgcgtttggctccacgctcgatccactggcgagtgttagtaacagcactgttgcttcgtagcggagcatgacggccgtgggaactcctccttggtaacaaggacccacggggccaaaagccacgcccacacgggcccgtcatgtgtgcaaccccagcacggcgactttactgcgaaacccactttaaagtgacattgaaactggtacccacacactggtgacaggctaaggatgcccttcaggtaccccgaggtaacacgcgacactcgggatctgagaaggggactggggcttctataaaagcgctcggtttaaaaagcttctatgcctgaataggtgaccggaggtcggcacctttcctttgcaattactgaccac

SEQ ID NO: 7 - DNA, 551 bp, Encephalomyocarditis virus
cgttactggccgaagccgcttggaataaggccggtgtgcgtttgtctatatgttattttccaccatattgccgtcttttggcaatgtgagggcccggaaacctggccctgtcttcttgacgagcattcctaggggtctttcccctctcgccaaaggaatgcaaggtctgttgaatgtcgtgaaggaagcagttcctctggaagcttcttgaagacaaacaacgtctgtagcgaccctttgcaggcagcggaaccccccacctggcgacaggtgcctctgcggccaaaagccacgtgtataagatacacctgcaaaggcggcacaaccccagtgccacgttgtgagttggatagttgtggaaagagtcaaatggctcccctcaagcgtattcaacaaggggctgaaggatgcccagaaggtaccccattgtatgggatctgatctggggcctcggtgcacatgcttttcatgtgtttagtcgaggttaaaaaacgtctaggccccccgaaccacggggacgtggttttcctttgaaaaacacgatgataata

SEQ ID NO: 8 - DNA, 84 bp, Unknown
  Viral 2A peptide spacer sequence
cgcgcgaaacgcgcgccggtgaaacagaccctgaactttgatctgctgaaactggcgggcgatgtggaaagcaacccgggcccg

SEQ ID NO: 9 - DNA, 45 bp, Unknown
  Flexible linker sequence.
ggaggtggcgggtccgggggcgggggtagcggtggcgggggctcc

SEQ ID NO: 10 - DNA, 592 bp, Woodchuck hepatitis virus
aatcaacctctggattacaaaatttgtgaaagattgactggtattcttaactatgttgctccttttacgctatgtggatacgctgctttaatgcctttgtatcatgctattgcttcccgtatggctttcattttctcctccttgtataaatcctggttgctgtctctttatgaggagttgtggcccgttgtcaggcaacgtggcgtggtgtgcactgtgtttgctgacgcaacccccactggttggggcattgccaccacctgtcagctcctttccgggactttcgctttccccctccctattgccacggcggaactcatcgccgcctgccttgcccgctgctggacaggggctcggctgttgggcactgacaattccgtggtgttgtcggggaagctgacgtcctttccatggctgctcgcctgtgttgccacctggattctgcgcgggacgtccttctgctacgtcccttcggccctcaatccagcggaccttccttcccgcggcctgctgccggctctgcggcctcttccgcgtcttcgccttcgccctcagacgagtcggatctccctttgggccgcctccccgcctg

SEQ ID NO: 11 - DNA, 247 bp, Woodchuck hepatitis virus
aatcaacctctggattacaaaatttgtgaaagattgactggtattcttaactatgttgctccttttacgctatgtggatacgctgctttaatgcctttgtatcatgctattgcttcccgtatggctttcattttctcctccttgtataaatcctggttagttcttgccacggcggaactcatcgccgcctgccttgcccgctgctggacaggggctcggctgttgggcactgacaattccgtggtgt

SEQ ID NO: 12 - DNA, 224 bp, Simian virus 40
agcagacatgataagatacattgatgagtttggacaaaccacaactagaatgcagtgaaaaaaatgctttatttgtgaaatttgtgatgctattgctttatttgtaaccattataagctgcaataaacaagttaacaacaacaattgcattcattttatgtttcaggttcagggggaggtgtgggaggttttttaaagcaagtaaaacctctacaaatgtggta

SEQ ID NO: 13 - DNA, 6633 bp, Unknown
  An embodiemnt of the AAAV1 vector of the invention, which includes a CMV promoter, a CMV enchancer, an EMCV IRES, and a SV40 poly A tail.
cctgcaggcagctgcgcgctcgctcgctcactgaggccgcccgggcgtcgggcgacctttggtcgcccggcctcagtgagcgagcgagcgcgcagagagggagtggccaactccatcactaggggttcctgcggccggtcgcgtactagtaatcaattacggggtcattagttcatagcccatatatggagttccgcgttacataacttacggtaaatggcccgcctggctgaccgcccaacgacccccgcccattgacgtcaataatgacgtatgttcccatagtaacgccaatagggactttccattgacgtcaatgggtggagtatttacggtaaactgcccacttggcagtacatcaagtgtatcatatgccaagtacgccccctattgacgtcaatgacggtaaatggcccgcctggcattatgcccagtacatgaccttatgggactttcctacttggcagtacatctacgtattagtcatcgctattaccatgctgatgcggttttggcagtacatcaatgggcgtggatagcggtttgactcacggggatttccaagtctccaccccattgacgtcaatgggagtttgttttggcaccaaaatcaacgggactttccaaaatgtcgtaacaactccgccccattgacgcaaatgggcggtaggcgtgtacggtgggaggtctatataagcagagctggtttagtgaaccgtcagatcagatctttgtcgatcctaccatccactcgacacacccgccagcggccgctgccaagcttccgagctctcgaattcaaaggaggtacccaccatggccaccatgagccccgcggggcccaaggtcccctggttcccaagaaaagtgtcagagctggacaagtgtcatcacctggtcaccaagttcgaccctgacctggacttggaccacccgggcttctcggaccaggtgtaccgccagcgcaggaagctgattgctgagatcgccttccagtacaggcacggcgacccgattccccgtgtggagtacaccgccgaggagattgccacctggaaggaggtctacaccacgctgaagggcctctacgccacgcacgcctgcggggagcacctggaggcctttgctttgctggagcgcttcagcggctaccgggaagacaatatcccccagctggaggacgtctcccgcttcctgaaggagcgcacgggcttccagctgcggcctgtggccggcctgctgtccgcccgggacttcctggccagcctggccttccgcgtgttccagtgcacccagtatatccgccacgcgtcctcgcccatgcactcccctgagccggactgctgccacgagctgctggggcacgtgcccatgctggccgaccgcaccttcgcgcagttctcgcaggacattggcctggcgtccctgggggcctcggatgaggaaattgagaagctgtccacgctgtactggttcacggtggagttcgggctgtgtaagcagaacggggaggtgaaggcctatggtgccgggctgctgtcctcctacggggagctcctgcactgcctgtctgaggagcctgagattcgggccttcgaccctgaggctgcggccgtgcagccctaccaagaccagacgtaccagtcagtctacttcgtgtctgagagcttcagtgacgccaaggacaagctcaggagctatgcctcacgcatccagcgccccttctccgtgaagttcgacccgtacacgctggccatcgacgtgctggacagcccccaggccgtgcggcgctccctggagggtgtccaggatgagctggacacccttgcccatgcgctgagtgccattggctaaacgttactggccgaagccgcttggaataaggccggtgtgcgtttgtctatatgttattttccaccatattgccgtcttttggcaatgtgagggcccggaaacctggccctgtcttcttgacgagcattcctaggggtctttcccctctcgccaaaggaatgcaaggtctgttgaatgtcgtgaaggaagcagttcctctggaagcttcttgaagacaaacaacgtctgtagcgaccctttgcaggcagcggaaccccccacctggcgacaggtgcctctgcggccaaaagccacgtgtataagatacacctgcaaaggcggcacaaccccagtgccacgttgtgagttggatagttgtggaaagagtcaaatggctcccctcaagcgtattcaacaaggggctgaaggatgcccagaaggtaccccattgtatgggatctgatctggggcctcggtgcacatgcttttcatgtgtttagtcgaggttaaaaaacgtctaggccccccgaaccacggggacgtggttttcctttgaaaaacacgatgataatagccaccatggagaagggccctgtgcgggcaccggcggagaagccgcggggcgccaggtgcagcaatgggttccccgagcgggatccgccgcggcccgggcccagcaggccggcggagaagcccccgcggcccgaggccaagagcgcgcagcccgcggacggctggaagggcgagcggccccgcagcgaggaggataacgagctgaacctccctaacctggcagccgcctactcgtccatcctgagctcgctgggcgagaacccccagcggcaagggctgctcaagacgccctggagggcggcctcggccatgcagttcttcaccaagggctaccaggagaccatctcagatgtcctaaacgatgctatatttgatgaagatcatgatgagatggtgattgtgaaggacatagacatgttttccatgtgtgagcatcacttggttccatttgttggaaaggtccatattggttatcttcctaacaagcaagtccttggcctcagcaaacttgcgaggattgtagaaatctatagtagaagactacaagttcaggagcgccttacaaaacaaattgctgtagcaatcacggaagccttgcggcctgctggagtcggggtagtggttgaagcaacacacatgtgtatggtaatgcgaggtgtacagaaaatgaacagcaaaactgtgaccagcacaatgttgggtgtgttccgggaggatccaaagactcgggaagagttcctgactctcattaggagctgagccacctaatcaacctctggattacaaaatttgtgaaagattgactggtattcttaactatgttgctccttttacgctatgtggatacgctgctttaatgcctttgtatcatgctattgcttcccgtatggctttcattttctcctccttgtataaatcctggttgctgtctctttatgaggagttgtggcccgttgtcaggcaacgtggcgtggtgtgcactgtgtttgctgacgcaacccccactggttggggcattgccaccacctgtcagctcctttccgggactttcgctttccccctccctattgccacggcggaactcatcgccgcctgccttgcccgctgctggacaggggctcggctgttgggcactgacaattccgtggtgttgtcggggaaatcatcgtcctttccctggctgactgatacaatcgatttctggatccgcaggcctctgctagcttgactgactgagatacagcgtaccttcagctcacagacatgataagatacattgatgagtttggacaaaccacaactagaatgcagtgaaaaaaatgctttatttgtgaaatttgtgatgctattgctttatttgtaaccattataagctgcaataaacaagttaacaacaacaattgcattcattttatgtttcaggttcagggggaggtgtgggaggttttttaagcttaacgcggtaaccacgtgcggacccaacggccgcaggaacccctagtgatggagttggccactccctctctgcgcgctcgctcgctcactgaggccgggcgaccaaaggtcgcccgacgcccgggctttgcccgggcggcctcagtgagcgagcgagcgcgcagctgcctgcaggggcgcctgatgcggtattttctccttacgcatctgtgcggtatttcacaccgcatacgtcaaagcaaccatagtacgcgccctgtagcggcgcattaagcgcggcgggtgtggtggttacgcgcagcgtgaccgctacacttgccagcgccctagcgcccgctcctttcgctttcttcccttcctttctcgccacgttcgccggctttccccgtcaagctctaaatcgggggctccctttagggttccgatttagtgctttacggcacctcgaccccaaaaaacttgatttgggtgatggttcacgtagtgggccatcgccctgatagacggtttttcgccctttgacgttggagtccacgttctttaatagtggactcttgttccaaactggaacaacactcaaccctatctcgggctattcttttgatttataagggattttgccgatttcggcctattggttaaaaaatgagctgatttaacaaaaatttaacgcgaattttaacaaaatattaacgtttacaattttatggtgcactctcagtacaatctgctctgatgccgcatagttaagccagccccgacacccgccaacacccgctgacgcgccctgacgggcttgtctgctcccggcatccgcttacagacaagctgtgaccgtctccgggagctgcatgtgtcagaggttttcaccgtcatcaccgaaacgcgcgagacgaaagggcctcgtgatacgcctatttttataggttaatgtcatgataataatggtttcttagacgtcaggtggcacttttcggggaaatgtgcgcggaacccctatttgtttatttttctaaatacattcaaatatgtatccgctcatgagacaataaccctgataaatgcttcaataatattgaaaaaggaagagtatgagtattcaacatttccgtgtcgcccttattcccttttttgcggcattttgccttcctgtttttgctcacccagaaacgctggtgaaagtaaaagatgctgaagatcagttgggtgcacgagtgggttacatcgaactggatctcaacagcggtaagatccttgagagttttcgccccgaagaacgttttccaatgatgagcacttttaaagttctgctatgtggcgcggtattatcccgtattgacgccgggcaagagcaactcggtcgccgcatacactattctcagaatgacttggttgagtactcaccagtcacagaaaagcatcttacggatggcatgacagtaagagaattatgcagtgctgccataaccatgagtgataacactgcggccaacttacttctgacaacgatcggaggaccgaaggagctaaccgcttttttgcacaacatgggggatcatgtaactcgccttgatcgttgggaaccggagctgaatgaagccataccaaacgacgagcgtgacaccacgatgcctgtagcaatggcaacaacgttgcgcaaactattaactggcgaactacttactctagcttcccggcaacaattaatagactggatggaggcggataaagttgcaggaccacttctgcgctcggcccttccggctggctggtttattgctgataaatctggagccggtgagcgtgggtctcgcggtatcattgcagcactggggccagatggtaagccctcccgtatcgtagttatctacacgacggggagtcaggcaactatggatgaacgaaatagacagatcgctgagataggtgcctcactgattaagcattggtaactgtcagaccaagtttactcatatatactttagattgatttaaaacttcatttttaatttaaaaggatctaggtgaagatcctttttgataatctcatgaccaaaatcccttaacgtgagttttcgttccactgagcgtcagaccccgtagaaaagatcaaaggatcttcttgagatcctttttttctgcgcgtaatctgctgcttgcaaacaaaaaaaccaccgctaccagcggtggtttgtttgccggatcaagagctaccaactctttttccgaaggtaactggcttcagcagagcgcagataccaaatactgtccttctagtgtagccgtagttaggccaccacttcaagaactctgtagcaccgcctacatacctcgctctgctaatcctgttaccagtggctgctgccagtggcgataagtcgtgtcttaccgggttggactcaagacgatagttaccggataaggcgcagcggtcgggctgaacggggggttcgtgcacacagcccagcttggagcgaacgacctacaccgaactgagatacctacagcgtgagctatgagaaagcgccacgcttcccgaagggagaaaggcggacaggtatccggtaagcggcagggtcggaacaggagagcgcacgagggagcttccagggggaaacgcctggtatctttatagtcctgtcgggtttcgccacctctgacttgagcgtcgatttttgtgatgctcgtcaggggggcggagcctatggaaaaacgccagcaacgcggcctttttacggttcctggccttttgctggccttttgctcacatgt

SEQ ID NO: 14 - DNA, 6542 bp, Unknown
  An example of a AAAV1 vector of the invention. Thjis vector similar to SEQ ID NO: 13, but this particular embodiment includes an FMDV IRES instead of the EMCV IRES.
cctgcaggcagctgcgcgctcgctcgctcactgaggccgcccgggcgtcgggcgacctttggtcgcccggcctcagtgagcgagcgagcgcgcagagagggagtggccaactccatcactaggggttcctgcggccggtcgcgtactagtaatcaattacggggtcattagttcatagcccatatatggagttccgcgttacataacttacggtaaatggcccgcctggctgaccgcccaacgacccccgcccattgacgtcaataatgacgtatgttcccatagtaacgccaatagggactttccattgacgtcaatgggtggagtatttacggtaaactgcccacttggcagtacatcaagtgtatcatatgccaagtacgccccctattgacgtcaatgacggtaaatggcccgcctggcattatgcccagtacatgaccttatgggactttcctacttggcagtacatctacgtattagtcatcgctattaccatgctgatgcggttttggcagtacatcaatgggcgtggatagcggtttgactcacggggatttccaagtctccaccccattgacgtcaatgggagtttgttttggcaccaaaatcaacgggactttccaaaatgtcgtaacaactccgccccattgacgcaaatgggcggtaggcgtgtacggtgggaggtctatataagcagagctggtttagtgaaccgtcagatcagatctttgtcgatcctaccatccactcgacacacccgccagcggccgctgccaagcttccgagctctcgaattcaaaggaggtacccaccatggccaccatgagccccgcggggcccaaggtcccctggttcccaagaaaagtgtcagagctggacaagtgtcatcacctggtcaccaagttcgaccctgacctggacttggaccacccgggcttctcggaccaggtgtaccgccagcgcaggaagctgattgctgagatcgccttccagtacaggcacggcgacccgattccccgtgtggagtacaccgccgaggagattgccacctggaaggaggtctacaccacgctgaagggcctctacgccacgcacgcctgcggggagcacctggaggcctttgctttgctggagcgcttcagcggctaccgggaagacaatatcccccagctggaggacgtctcccgcttcctgaaggagcgcacgggcttccagctgcggcctgtggccggcctgctgtccgcccgggacttcctggccagcctggccttccgcgtgttccagtgcacccagtatatccgccacgcgtcctcgcccatgcactcccctgagccggactgctgccacgagctgctggggcacgtgcccatgctggccgaccgcaccttcgcgcagttctcgcaggacattggcctggcgtccctgggggcctcggatgaggaaattgagaagctgtccacgctgtactggttcacggtggagttcgggctgtgtaagcagaacggggaggtgaaggcctatggtgccgggctgctgtcctcctacggggagctcctgcactgcctgtctgaggagcctgagattcgggccttcgaccctgaggctgcggccgtgcagccctaccaagaccagacgtaccagtcagtctacttcgtgtctgagagcttcagtgacgccaaggacaagctcaggagctatgcctcacgcatccagcgccccttctccgtgaagttcgacccgtacacgctggccatcgacgtgctggacagcccccaggccgtgcggcgctccctggagggtgtccaggatgagctggacacccttgcccatgcgctgagtgccattggctaaagcaggtttccccaactgacacaaaacgtgcaacttgaaactccgcctggtctttccaggtctagaggggtaacactttgtactgcgtttggctccacgctcgatccactggcgagtgttagtaacagcactgttgcttcgtagcggagcatgacggccgtgggaactcctccttggtaacaaggacccacggggccaaaagccacgcccacacgggcccgtcatgtgtgcaaccccagcacggcgactttactgcgaaacccactttaaagtgacattgaaactggtacccacacactggtgacaggctaaggatgcccttcaggtaccccgaggtaacacgcgacactcgggatctgagaaggggactggggcttctataaaagcgctcggtttaaaaagcttctatgcctgaataggtgaccggaggtcggcacctttcctttgcaattactgaccacgccaccatggagaagggccctgtgcgggcaccggcggagaagccgcggggcgccaggtgcagcaatgggttccccgagcgggatccgccgcggcccgggcccagcaggccggcggagaagcccccgcggcccgaggccaagagcgcgcagcccgcggacggctggaagggcgagcggccccgcagcgaggaggataacgagctgaacctccctaacctggcagccgcctactcgtccatcctgagctcgctgggcgagaacccccagcggcaagggctgctcaagacgccctggagggcggcctcggccatgcagttcttcaccaagggctaccaggagaccatctcagatgtcctaaacgatgctatatttgatgaagatcatgatgagatggtgattgtgaaggacatagacatgttttccatgtgtgagcatcacttggttccatttgttggaaaggtccatattggttatcttcctaacaagcaagtccttggcctcagcaaacttgcgaggattgtagaaatctatagtagaagactacaagttcaggagcgccttacaaaacaaattgctgtagcaatcacggaagccttgcggcctgctggagtcggggtagtggttgaagcaacacacatgtgtatggtaatgcgaggtgtacagaaaatgaacagcaaaactgtgaccagcacaatgttgggtgtgttccgggaggatccaaagactcgggaagagttcctgactctcattaggagctgagccacctaatcaacctctggattacaaaatttgtgaaagattgactggtattcttaactatgttgctccttttacgctatgtggatacgctgctttaatgcctttgtatcatgctattgcttcccgtatggctttcattttctcctccttgtataaatcctggttgctgtctctttatgaggagttgtggcccgttgtcaggcaacgtggcgtggtgtgcactgtgtttgctgacgcaacccccactggttggggcattgccaccacctgtcagctcctttccgggactttcgctttccccctccctattgccacggcggaactcatcgccgcctgccttgcccgctgctggacaggggctcggctgttgggcactgacaattccgtggtgttgtcggggaaatcatcgtcctttccctggctgactgatacaatcgatttctggatccgcaggcctctgctagcttgactgactgagatacagcgtaccttcagctcacagacatgataagatacattgatgagtttggacaaaccacaactagaatgcagtgaaaaaaatgctttatttgtgaaatttgtgatgctattgctttatttgtaaccattataagctgcaataaacaagttaacaacaacaattgcattcattttatgtttcaggttcagggggaggtgtgggaggttttttaagcttaacgcggtaaccacgtgcggacccaacggccgcaggaacccctagtgatggagttggccactccctctctgcgcgctcgctcgctcactgaggccgggcgaccaaaggtcgcccgacgcccgggctttgcccgggcggcctcagtgagcgagcgagcgcgcagctgcctgcaggggcgcctgatgcggtattttctccttacgcatctgtgcggtatttcacaccgcatacgtcaaagcaaccatagtacgcgccctgtagcggcgcattaagcgcggcgggtgtggtggttacgcgcagcgtgaccgctacacttgccagcgccctagcgcccgctcctttcgctttcttcccttcctttctcgccacgttcgccggctttccccgtcaagctctaaatcgggggctccctttagggttccgatttagtgctttacggcacctcgaccccaaaaaacttgatttgggtgatggttcacgtagtgggccatcgccctgatagacggtttttcgccctttgacgttggagtccacgttctttaatagtggactcttgttccaaactggaacaacactcaaccctatctcgggctattcttttgatttataagggattttgccgatttcggcctattggttaaaaaatgagctgatttaacaaaaatttaacgcgaattttaacaaaatattaacgtttacaattttatggtgcactctcagtacaatctgctctgatgccgcatagttaagccagccccgacacccgccaacacccgctgacgcgccctgacgggcttgtctgctcccggcatccgcttacagacaagctgtgaccgtctccgggagctgcatgtgtcagaggttttcaccgtcatcaccgaaacgcgcgagacgaaagggcctcgtgatacgcctatttttataggttaatgtcatgataataatggtttcttagacgtcaggtggcacttttcggggaaatgtgcgcggaacccctatttgtttatttttctaaatacattcaaatatgtatccgctcatgagacaataaccctgataaatgcttcaataatattgaaaaaggaagagtatgagtattcaacatttccgtgtcgcccttattcccttttttgcggcattttgccttcctgtttttgctcacccagaaacgctggtgaaagtaaaagatgctgaagatcagttgggtgcacgagtgggttacatcgaactggatctcaacagcggtaagatccttgagagttttcgccccgaagaacgttttccaatgatgagcacttttaaagttctgctatgtggcgcggtattatcccgtattgacgccgggcaagagcaactcggtcgccgcatacactattctcagaatgacttggttgagtactcaccagtcacagaaaagcatcttacggatggcatgacagtaagagaattatgcagtgctgccataaccatgagtgataacactgcggccaacttacttctgacaacgatcggaggaccgaaggagctaaccgcttttttgcacaacatgggggatcatgtaactcgccttgatcgttgggaaccggagctgaatgaagccataccaaacgacgagcgtgacaccacgatgcctgtagcaatggcaacaacgttgcgcaaactattaactggcgaactacttactctagcttcccggcaacaattaatagactggatggaggcggataaagttgcaggaccacttctgcgctcggcccttccggctggctggtttattgctgataaatctggagccggtgagcgtgggtctcgcggtatcattgcagcactggggccagatggtaagccctcccgtatcgtagttatctacacgacggggagtcaggcaactatggatgaacgaaatagacagatcgctgagataggtgcctcactgattaagcattggtaactgtcagaccaagtttactcatatatactttagattgatttaaaacttcatttttaatttaaaaggatctaggtgaagatcctttttgataatctcatgaccaaaatcccttaacgtgagttttcgttccactgagcgtcagaccccgtagaaaagatcaaaggatcttcttgagatcctttttttctgcgcgtaatctgctgcttgcaaacaaaaaaaccaccgctaccagcggtggtttgtttgccggatcaagagctaccaactctttttccgaaggtaactggcttcagcagagcgcagataccaaatactgtccttctagtgtagccgtagttaggccaccacttcaagaactctgtagcaccgcctacatacctcgctctgctaatcctgttaccagtggctgctgccagtggcgataagtcgtgtcttaccgggttggactcaagacgatagttaccggataaggcgcagcggtcgggctgaacggggggttcgtgcacacagcccagcttggagcgaacgacctacaccgaactgagatacctacagcgtgagctatgagaaagcgccacgcttcccgaagggagaaaggcggacaggtatccggtaagcggcagggtcggaacaggagagcgcacgagggagcttccagggggaaacgcctggtatctttatagtcctgtcgggtttcgccacctctgacttgagcgtcgatttttgtgatgctcgtcaggggggcggagcctatggaaaaacgccagcaacgcggcctttttacggttcctggccttttgctggccttttgctcacatgt

SEQ ID NO: 15 - DNA, 6165 bp, Unknown
  An example of an AAAV1 vector of the invention. This is similar to SEQ ID NO: 13, but this particular embodiment includes a Furin cleavage site and a viral 2A peptide spacer, instead of the EMCV IRES
cctgcaggcagctgcgcgctcgctcgctcactgaggccgcccgggcgtcgggcgacctttggtcgcccggcctcagtgagcgagcgagcgcgcagagagggagtggccaactccatcactaggggttcctgcggccggtcgcgtactagtaatcaattacggggtcattagttcatagcccatatatggagttccgcgttacataacttacggtaaatggcccgcctggctgaccgcccaacgacccccgcccattgacgtcaataatgacgtatgttcccatagtaacgccaatagggactttccattgacgtcaatgggtggagtatttacggtaaactgcccacttggcagtacatcaagtgtatcatatgccaagtacgccccctattgacgtcaatgacggtaaatggcccgcctggcattatgcccagtacatgaccttatgggactttcctacttggcagtacatctacgtattagtcatcgctattaccatgctgatgcggttttggcagtacatcaatgggcgtggatagcggtttgactcacggggatttccaagtctccaccccattgacgtcaatgggagtttgttttggcaccaaaatcaacgggactttccaaaatgtcgtaacaactccgccccattgacgcaaatgggcggtaggcgtgtacggtgggaggtctatataagcagagctggtttagtgaaccgtcagatcagatctttgtcgatcctaccatccactcgacacacccgccagcggccgctgccaagcttccgagctctcgaattcaaaggaggtacccaccatggccaccatgagccccgcggggcccaaggtcccctggttcccaagaaaagtgtcagagctggacaagtgtcatcacctggtcaccaagttcgaccctgacctggacttggaccacccgggcttctcggaccaggtgtaccgccagcgcaggaagctgattgctgagatcgccttccagtacaggcacggcgacccgattccccgtgtggagtacaccgccgaggagattgccacctggaaggaggtctacaccacgctgaagggcctctacgccacgcacgcctgcggggagcacctggaggcctttgctttgctggagcgcttcagcggctaccgggaagacaatatcccccagctggaggacgtctcccgcttcctgaaggagcgcacgggcttccagctgcggcctgtggccggcctgctgtccgcccgggacttcctggccagcctggccttccgcgtgttccagtgcacccagtatatccgccacgcgtcctcgcccatgcactcccctgagccggactgctgccacgagctgctggggcacgtgcccatgctggccgaccgcaccttcgcgcagttctcgcaggacattggcctggcgtccctgggggcctcggatgaggaaattgagaagctgtccacgctgtactggttcacggtggagttcgggctgtgtaagcagaacggggaggtgaaggcctatggtgccgggctgctgtcctcctacggggagctcctgcactgcctgtctgaggagcctgagattcgggccttcgaccctgaggctgcggccgtgcagccctaccaagaccagacgtaccagtcagtctacttcgtgtctgagagcttcagtgacgccaaggacaagctcaggagctatgcctcacgcatccagcgccccttctccgtgaagttcgacccgtacacgctggccatcgacgtgctggacagcccccaggccgtgcggcgctccctggagggtgtccaggatgagctggacacccttgcccatgcgctgagtgccattggctaacgcgcgaaacgcgcgccggtgaaacagaccctgaactttgatctgctgaaactggcgggcgatgtggaaagcaacccgggcccggccaccatggagaagggccctgtgcgggcaccggcggagaagccgcggggcgccaggtgcagcaatgggttccccgagcgggatccgccgcggcccgggcccagcaggccggcggagaagcccccgcggcccgaggccaagagcgcgcagcccgcggacggctggaagggcgagcggccccgcagcgaggaggataacgagctgaacctccctaacctggcagccgcctactcgtccatcctgagctcgctgggcgagaacccccagcggcaagggctgctcaagacgccctggagggcggcctcggccatgcagttcttcaccaagggctaccaggagaccatctcagatgtcctaaacgatgctatatttgatgaagatcatgatgagatggtgattgtgaaggacatagacatgttttccatgtgtgagcatcacttggttccatttgttggaaaggtccatattggttatcttcctaacaagcaagtccttggcctcagcaaacttgcgaggattgtagaaatctatagtagaagactacaagttcaggagcgccttacaaaacaaattgctgtagcaatcacggaagccttgcggcctgctggagtcggggtagtggttgaagcaacacacatgtgtatggtaatgcgaggtgtacagaaaatgaacagcaaaactgtgaccagcacaatgttgggtgtgttccgggaggatccaaagactcgggaagagttcctgactctcattaggagctgagccacctaatcaacctctggattacaaaatttgtgaaagattgactggtattcttaactatgttgctccttttacgctatgtggatacgctgctttaatgcctttgtatcatgctattgcttcccgtatggctttcattttctcctccttgtataaatcctggttgctgtctctttatgaggagttgtggcccgttgtcaggcaacgtggcgtggtgtgcactgtgtttgctgacgcaacccccactggttggggcattgccaccacctgtcagctcctttccgggactttcgctttccccctccctattgccacggcggaactcatcgccgcctgccttgcccgctgctggacaggggctcggctgttgggcactgacaattccgtggtgttgtcggggaaatcatcgtcctttccctggctgactgatacaatcgatttctggatccgcaggcctctgctagcttgactgactgagatacagcgtaccttcagctcacagacatgataagatacattgatgagtttggacaaaccacaactagaatgcagtgaaaaaaatgctttatttgtgaaatttgtgatgctattgctttatttgtaaccattataagctgcaataaacaagttaacaacaacaattgcattcattttatgtttcaggttcagggggaggtgtgggaggttttttaagcttaacgcggtaaccacgtgcggacccaacggccgcaggaacccctagtgatggagttggccactccctctctgcgcgctcgctcgctcactgaggccgggcgaccaaaggtcgcccgacgcccgggctttgcccgggcggcctcagtgagcgagcgagcgcgcagctgcctgcaggggcgcctgatgcggtattttctccttacgcatctgtgcggtatttcacaccgcatacgtcaaagcaaccatagtacgcgccctgtagcggcgcattaagcgcggcgggtgtggtggttacgcgcagcgtgaccgctacacttgccagcgccctagcgcccgctcctttcgctttcttcccttcctttctcgccacgttcgccggctttccccgtcaagctctaaatcgggggctccctttagggttccgatttagtgctttacggcacctcgaccccaaaaaacttgatttgggtgatggttcacgtagtgggccatcgccctgatagacggtttttcgccctttgacgttggagtccacgttctttaatagtggactcttgttccaaactggaacaacactcaaccctatctcgggctattcttttgatttataagggattttgccgatttcggcctattggttaaaaaatgagctgatttaacaaaaatttaacgcgaattttaacaaaatattaacgtttacaattttatggtgcactctcagtacaatctgctctgatgccgcatagttaagccagccccgacacccgccaacacccgctgacgcgccctgacgggcttgtctgctcccggcatccgcttacagacaagctgtgaccgtctccgggagctgcatgtgtcagaggttttcaccgtcatcaccgaaacgcgcgagacgaaagggcctcgtgatacgcctatttttataggttaatgtcatgataataatggtttcttagacgtcaggtggcacttttcggggaaatgtgcgcggaacccctatttgtttatttttctaaatacattcaaatatgtatccgctcatgagacaataaccctgataaatgcttcaataatattgaaaaaggaagagtatgagtattcaacatttccgtgtcgcccttattcccttttttgcggcattttgccttcctgtttttgctcacccagaaacgctggtgaaagtaaaagatgctgaagatcagttgggtgcacgagtgggttacatcgaactggatctcaacagcggtaagatccttgagagttttcgccccgaagaacgttttccaatgatgagcacttttaaagttctgctatgtggcgcggtattatcccgtattgacgccgggcaagagcaactcggtcgccgcatacactattctcagaatgacttggttgagtactcaccagtcacagaaaagcatcttacggatggcatgacagtaagagaattatgcagtgctgccataaccatgagtgataacactgcggccaacttacttctgacaacgatcggaggaccgaaggagctaaccgcttttttgcacaacatgggggatcatgtaactcgccttgatcgttgggaaccggagctgaatgaagccataccaaacgacgagcgtgacaccacgatgcctgtagcaatggcaacaacgttgcgcaaactattaactggcgaactacttactctagcttcccggcaacaattaatagactggatggaggcggataaagttgcaggaccacttctgcgctcggcccttccggctggctggtttattgctgataaatctggagccggtgagcgtgggtctcgcggtatcattgcagcactggggccagatggtaagccctcccgtatcgtagttatctacacgacggggagtcaggcaactatggatgaacgaaatagacagatcgctgagataggtgcctcactgattaagcattggtaactgtcagaccaagtttactcatatatactttagattgatttaaaacttcatttttaatttaaaaggatctaggtgaagatcctttttgataatctcatgaccaaaatcccttaacgtgagttttcgttccactgagcgtcagaccccgtagaaaagatcaaaggatcttcttgagatcctttttttctgcgcgtaatctgctgcttgcaaacaaaaaaaccaccgctaccagcggtggtttgtttgccggatcaagagctaccaactctttttccgaaggtaactggcttcagcagagcgcagataccaaatactgtccttctagtgtagccgtagttaggccaccacttcaagaactctgtagcaccgcctacatacctcgctctgctaatcctgttaccagtggctgctgccagtggcgataagtcgtgtcttaccgggttggactcaagacgatagttaccggataaggcgcagcggtcgggctgaacggggggttcgtgcacacagcccagcttggagcgaacgacctacaccgaactgagatacctacagcgtgagctatgagaaagcgccacgcttcccgaagggagaaaggcggacaggtatccggtaagcggcagggtcggaacaggagagcgcacgagggagcttccagggggaaacgcctggtatctttatagtcctgtcgggtttcgccacctctgacttgagcgtcgatttttgtgatgctcgtcaggggggcggagcctatggaaaaacgccagcaacgcggcctttttacggttcctggccttttgctggccttttgctcacatgt

SEQ ID NO: 16 - DNA, 6126 bp, Unknown
  An example of an AAAV1 vector of the invention. This is similar to SEQ ID NO: 13, but this particular embodiment includes a flexible linker, instead of the EMCV IRES.
cctgcaggcagctgcgcgctcgctcgctcactgaggccgcccgggcgtcgggcgacctttggtcgcccggcctcagtgagcgagcgagcgcgcagagagggagtggccaactccatcactaggggttcctgcggccggtcgcgtactagtaatcaattacggggtcattagttcatagcccatatatggagttccgcgttacataacttacggtaaatggcccgcctggctgaccgcccaacgacccccgcccattgacgtcaataatgacgtatgttcccatagtaacgccaatagggactttccattgacgtcaatgggtggagtatttacggtaaactgcccacttggcagtacatcaagtgtatcatatgccaagtacgccccctattgacgtcaatgacggtaaatggcccgcctggcattatgcccagtacatgaccttatgggactttcctacttggcagtacatctacgtattagtcatcgctattaccatgctgatgcggttttggcagtacatcaatgggcgtggatagcggtttgactcacggggatttccaagtctccaccccattgacgtcaatgggagtttgttttggcaccaaaatcaacgggactttccaaaatgtcgtaacaactccgccccattgacgcaaatgggcggtaggcgtgtacggtgggaggtctatataagcagagctggtttagtgaaccgtcagatcagatctttgtcgatcctaccatccactcgacacacccgccagcggccgctgccaagcttccgagctctcgaattcaaaggaggtacccaccatggccaccatgagccccgcggggcccaaggtcccctggttcccaagaaaagtgtcagagctggacaagtgtcatcacctggtcaccaagttcgaccctgacctggacttggaccacccgggcttctcggaccaggtgtaccgccagcgcaggaagctgattgctgagatcgccttccagtacaggcacggcgacccgattccccgtgtggagtacaccgccgaggagattgccacctggaaggaggtctacaccacgctgaagggcctctacgccacgcacgcctgcggggagcacctggaggcctttgctttgctggagcgcttcagcggctaccgggaagacaatatcccccagctggaggacgtctcccgcttcctgaaggagcgcacgggcttccagctgcggcctgtggccggcctgctgtccgcccgggacttcctggccagcctggccttccgcgtgttccagtgcacccagtatatccgccacgcgtcctcgcccatgcactcccctgagccggactgctgccacgagctgctggggcacgtgcccatgctggccgaccgcaccttcgcgcagttctcgcaggacattggcctggcgtccctgggggcctcggatgaggaaattgagaagctgtccacgctgtactggttcacggtggagttcgggctgtgtaagcagaacggggaggtgaaggcctatggtgccgggctgctgtcctcctacggggagctcctgcactgcctgtctgaggagcctgagattcgggccttcgaccctgaggctgcggccgtgcagccctaccaagaccagacgtaccagtcagtctacttcgtgtctgagagcttcagtgacgccaaggacaagctcaggagctatgcctcacgcatccagcgccccttctccgtgaagttcgacccgtacacgctggccatcgacgtgctggacagcccccaggccgtgcggcgctccctggagggtgtccaggatgagctggacacccttgcccatgcgctgagtgccattggctaaggaggtggcgggtccgggggcgggggtagcggtggcgggggctccgccaccatggagaagggccctgtgcgggcaccggcggagaagccgcggggcgccaggtgcagcaatgggttccccgagcgggatccgccgcggcccgggcccagcaggccggcggagaagcccccgcggcccgaggccaagagcgcgcagcccgcggacggctggaagggcgagcggccccgcagcgaggaggataacgagctgaacctccctaacctggcagccgcctactcgtccatcctgagctcgctgggcgagaacccccagcggcaagggctgctcaagacgccctggagggcggcctcggccatgcagttcttcaccaagggctaccaggagaccatctcagatgtcctaaacgatgctatatttgatgaagatcatgatgagatggtgattgtgaaggacatagacatgttttccatgtgtgagcatcacttggttccatttgttggaaaggtccatattggttatcttcctaacaagcaagtccttggcctcagcaaacttgcgaggattgtagaaatctatagtagaagactacaagttcaggagcgccttacaaaacaaattgctgtagcaatcacggaagccttgcggcctgctggagtcggggtagtggttgaagcaacacacatgtgtatggtaatgcgaggtgtacagaaaatgaacagcaaaactgtgaccagcacaatgttgggtgtgttccgggaggatccaaagactcgggaagagttcctgactctcattaggagctgagccacctaatcaacctctggattacaaaatttgtgaaagattgactggtattcttaactatgttgctccttttacgctatgtggatacgctgctttaatgcctttgtatcatgctattgcttcccgtatggctttcattttctcctccttgtataaatcctggttgctgtctctttatgaggagttgtggcccgttgtcaggcaacgtggcgtggtgtgcactgtgtttgctgacgcaacccccactggttggggcattgccaccacctgtcagctcctttccgggactttcgctttccccctccctattgccacggcggaactcatcgccgcctgccttgcccgctgctggacaggggctcggctgttgggcactgacaattccgtggtgttgtcggggaaatcatcgtcctttccctggctgactgatacaatcgatttctggatccgcaggcctctgctagcttgactgactgagatacagcgtaccttcagctcacagacatgataagatacattgatgagtttggacaaaccacaactagaatgcagtgaaaaaaatgctttatttgtgaaatttgtgatgctattgctttatttgtaaccattataagctgcaataaacaagttaacaacaacaattgcattcattttatgtttcaggttcagggggaggtgtgggaggttttttaagcttaacgcggtaaccacgtgcggacccaacggccgcaggaacccctagtgatggagttggccactccctctctgcgcgctcgctcgctcactgaggccgggcgaccaaaggtcgcccgacgcccgggctttgcccgggcggcctcagtgagcgagcgagcgcgcagctgcctgcaggggcgcctgatgcggtattttctccttacgcatctgtgcggtatttcacaccgcatacgtcaaagcaaccatagtacgcgccctgtagcggcgcattaagcgcggcgggtgtggtggttacgcgcagcgtgaccgctacacttgccagcgccctagcgcccgctcctttcgctttcttcccttcctttctcgccacgttcgccggctttccccgtcaagctctaaatcgggggctccctttagggttccgatttagtgctttacggcacctcgaccccaaaaaacttgatttgggtgatggttcacgtagtgggccatcgccctgatagacggtttttcgccctttgacgttggagtccacgttctttaatagtggactcttgttccaaactggaacaacactcaaccctatctcgggctattcttttgatttataagggattttgccgatttcggcctattggttaaaaaatgagctgatttaacaaaaatttaacgcgaattttaacaaaatattaacgtttacaattttatggtgcactctcagtacaatctgctctgatgccgcatagttaagccagccccgacacccgccaacacccgctgacgcgccctgacgggcttgtctgctcccggcatccgcttacagacaagctgtgaccgtctccgggagctgcatgtgtcagaggttttcaccgtcatcaccgaaacgcgcgagacgaaagggcctcgtgatacgcctatttttataggttaatgtcatgataataatggtttcttagacgtcaggtggcacttttcggggaaatgtgcgcggaacccctatttgtttatttttctaaatacattcaaatatgtatccgctcatgagacaataaccctgataaatgcttcaataatattgaaaaaggaagagtatgagtattcaacatttccgtgtcgcccttattcccttttttgcggcattttgccttcctgtttttgctcacccagaaacgctggtgaaagtaaaagatgctgaagatcagttgggtgcacgagtgggttacatcgaactggatctcaacagcggtaagatccttgagagttttcgccccgaagaacgttttccaatgatgagcacttttaaagttctgctatgtggcgcggtattatcccgtattgacgccgggcaagagcaactcggtcgccgcatacactattctcagaatgacttggttgagtactcaccagtcacagaaaagcatcttacggatggcatgacagtaagagaattatgcagtgctgccataaccatgagtgataacactgcggccaacttacttctgacaacgatcggaggaccgaaggagctaaccgcttttttgcacaacatgggggatcatgtaactcgccttgatcgttgggaaccggagctgaatgaagccataccaaacgacgagcgtgacaccacgatgcctgtagcaatggcaacaacgttgcgcaaactattaactggcgaactacttactctagcttcccggcaacaattaatagactggatggaggcggataaagttgcaggaccacttctgcgctcggcccttccggctggctggtttattgctgataaatctggagccggtgagcgtgggtctcgcggtatcattgcagcactggggccagatggtaagccctcccgtatcgtagttatctacacgacggggagtcaggcaactatggatgaacgaaatagacagatcgctgagataggtgcctcactgattaagcattggtaactgtcagaccaagtttactcatatatactttagattgatttaaaacttcatttttaatttaaaaggatctaggtgaagatcctttttgataatctcatgaccaaaatcccttaacgtgagttttcgttccactgagcgtcagaccccgtagaaaagatcaaaggatcttcttgagatcctttttttctgcgcgtaatctgctgcttgcaaacaaaaaaaccaccgctaccagcggtggtttgtttgccggatcaagagctaccaactctttttccgaaggtaactggcttcagcagagcgcagataccaaatactgtccttctagtgtagccgtagttaggccaccacttcaagaactctgtagcaccgcctacatacctcgctctgctaatcctgttaccagtggctgctgccagtggcgataagtcgtgtcttaccgggttggactcaagacgatagttaccggataaggcgcagcggtcgggctgaacggggggttcgtgcacacagcccagcttggagcgaacgacctacaccgaactgagatacctacagcgtgagctatgagaaagcgccacgcttcccgaagggagaaaggcggacaggtatccggtaagcggcagggtcggaacaggagagcgcacgagggagcttccagggggaaacgcctggtatctttatagtcctgtcgggtttcgccacctctgacttgagcgtcgatttttgtgatgctcgtcaggggggcggagcctatggaaaaacgccagcaacgcggcctttttacggttcctggccttttgctggccttttgctcacatgt

SEQ ID NO: 17 - DNA, 4561 bp, Unknown
  A vector carrying AAV2 right and left ITRs. This vector is suitable for the production of AAV vectors.
cctgcaggcagctgcgcgctcgctcgctcactgaggccgcccgggcgtcgggcgacctttggtcgcccggcctcagtgagcgagcgagcgcgcagagagggagtggccaactccatcactaggggttcctgcggccggtcgcgtctagttattaatagtaatcaattacggggtcattagttcatagcccatatatggagttccgcgttacataacttacggtaaatggcccgcctggctgaccgcccaacgacccccgcccattgacgtcaataatgacgtatgttcccatagtaacgcaatagggactttccattgacgtcaatgggtggagtatttacggtaaactgcccacttggcagtacatcaagtgtatcatatgccaagtacgccccctattgacgtcaatgacggtaaatggcccgcctggcattatgcccagtacatgaccttatgggactttcctacttggcagtacatctacgtattagtcatcgctattaccatggtgatgcggttttggcagtacatcaatgggcgtggatagcggtttgactcacggggatttccaagtctccaccccattgacgtcaatgggagtttgttttgcaccaaaatcaacgggactttccaaaatgtcgtaacaactccgccccattgacgcaaatgggcggtaggcgtgtacggtgggaggtctatataagcagagctgtttagtgaaccgtcagatcgcctggagacgccatccacgctgttttgacctccatagaagacaccgggaccgatccagcctccgcggattcgaatcccggccgggaacggtgcattggaacgcggattccccgtgccaagagtgacgtaagtaccgcctatagagtctataggcccacaaaaaatgctttcttcttttaatatacttttttgtttatcttatttctaatactttccctaatctctttctttcagggcaataatgatacaatgtatcatgcctctttgcaccattctaaagaataacagtgataatttctgggttaaggcaatagcaatatttctgcatataaatatttctgcatataaattgtaactgatgtaagaggtttcatattgctaatagcagctacaatccagctaccattctgcttttattttatggttgggataaggctggattattctgagtccaagctaggcccttttgctaatcatgttcatacctcttatcttcctcccacagctcctgggcaacgtgctggtctgtgtgctggcccatcactttggcaaagaattgggattcgaacatcgattgaattcagatccgctagtaatacgactcactatagggagaggatccggtaccgaggagatctgccgccgcgatcgccggcgcgccagatctcacgcttaactagctagcggaccgacgcgtacgcggccgctcgaggattataaggatgacgacgataaattcgtcgagcaccaccaccaccaccactaataaggtttatccgatccaccggatctagataagatatccgatccaccggatctagataactgatcataatcagccataccacatttgtagaggttttacttgctttaaaaaacctcccacacctccccctgaacctgaaacataaaatgaatgcaattgttgttgttaacttgtttattgcagcttataatggttacaaataaagcaatagcatcacaaatttcacaaataaagcatttttttcactgcattctagttgtggtttgtccaaactcatcaatgtatcttaacgcggtaaccacgtgcggacccaacggccgcaggaacccctagtgatggagttggccactccctctagagctgcgcgctcgctcgctcactgaggccgggcgaccaaaggtcgcccgacgcccgggctttgcccgggcggcctcagtgagcgagcgagcgcgcagctgcctgcaggggcgcctgatgcggtattttctccttacgcatctgtgcggtatttcacaccgcatacgtcaaagcaaccatagtacgcgccctgtagcggcgcattaagcgcggcgggtgtggtggttacgcgcagcgtgaccgctacacttgccagcgccctagcgcccgctcctttcgctttcttcccttcctttctcgccacgttcgccggctttccccgtcaagctctaaatcgggggctccctttagggttccgatttagtgctttacggcacctcgaccccaaaaaacttgatttgggtgatggttcacgtagtgggccatcgccctgatagacggtttttcgccctttgacgttggagtccacgttctttaatagtggactcttgttccaaactggaacaacactcaaccctatctcgggctattcttttgatttataagggattttgccgatttcggcctattggttaaaaaatgagctgatttaacaaaaatttaacgcgaattttaacaaaatattaacgtttacaattttatggtgcactctcagtacaatctgctctgatgccgcatagttaagccagccccgacacccgccaacacccgctgacgcgccctgacgggcttgtctgctcccggcatccgcttacagacaagctgtgaccgtctccgggagctgcatgtgtcagaggttttcaccgtcatcaccgaaacgcgcgagacgaaagggcctcgtgatacgcctatttttataggttaatgtcatgataataatggtttcttagacgtcaggtggcacttttcggggaaatgtgcgcggaacccctatttgtttatttttctaaatacattcaaatatgtatccgctcatgagacaataaccctgataaatgcttcaataatattgaaaaaggaagagtatgagtattcaacatttccgtgtcgcccttattcccttttttgcggcattttgccttcctgtttttgctcacccagaaacgctggtgaaagtaaaagatgctgaagatcagttgggtgcacgagtgggttacatcgaactggatctcaacagcggtaagatccttgagagttttcgccccgaagaacgttttccaatgatgagcacttttaaagttctgctatgtggcgcggtattatcccgtattgacgccgggcaagagcaactcggtcgccgcatacactattctcagaatgacttggttgagtactcaccagtcacagaaaagcatcttacggatggcatgacagtaagagaattatgcagtgctgccataaccatgagtgataacactgcggccaacttacttctgacaacgatcggaggaccgaaggagctaaccgcttttttgcacaacatgggggatcatgtaactcgccttgatcgttgggaaccggagctgaatgaagccataccaaacgacgagcgtgacaccacgatgcctgtagcaatggcaacaacgttgcgcaaactattaactggcgaactacttactctagcttcccggcaacaattaatagactggatggaggcggataaagttgcaggaccacttctgcgctcggcccttccggctggctggtttattgctgataaatctggagccggtgagcgtgggtctcgcggtatcattgcagcactggggccagatggtaagccctcccgtatcgtagttatctacacgacggggagtcaggcaactatggatgaacgaaatagacagatcgctgagataggtgcctcactgattaagcattggtaactgtcagaccaagtttactcatatatactttagattgatttaaaacttcatttttaatttaaaaggatctaggtgaagatcctttttgataatctcatgaccaaaatcccttaacgtgagttttcgttccactgagcgtcagaccccgtagaaaagatcaaaggatcttcttgagatcctttttttctgcgcgtaatctgctgcttgcaaacaaaaaaaccaccgctaccagcggtggtttgtttgccggatcaagagctaccaactctttttccgaaggtaactggcttcagcagagcgcagataccaaatactgtccttctagtgtagccgtagttaggccaccacttcaagaactctgtagcaccgcctacatacctcgctctgctaatcctgttaccagtggctgctgccagtggcgataagtcgtgtcttaccgggttggactcaagacgatagttaccggataaggcgcagcggtcgggctgaacggggggttcgtgcacacagcccagcttggagcgaacgacctacaccgaactgagatacctacagcgtgagctatgagaaagcgccacgcttcccgaagggagaaaggcggacaggtatccggtaagcggcagggtcggaacaggagagcgcacgagggagcttccagggggaaacgcctggtatctttatagtcctgtcgggtttcgccacctctgacttgagcgtcgatttttgtgatgctcgtcaggggggcggagcctatggaaaaacgccagcaacgcggcctttttacggttcctggccttttgctggccttttgctcacatgt

SEQ ID NO: 18 - DNA, 6773 bp, Unknown
  The genetic construct as shown in Fig. 10, which includes a CMV promoter and murine GCH1.
ggcgatcgcggctcccgacatcttggaccattagctccacaggtatcttcttccctctagtggtcataacagcagcttcagctacctctcaattcaaaaaacccctcaagacccgtttagaggccccaaggggttatgctatcaatcgttgcgttacacacacaaaaaaccaacacacatccatcttcgatggatagcgattttattatctaactgctgatcgagtgtagccagatctagtaatcaattacggggtcattagttcatagcccatatatggagttccgcgttacataacttacggtaaatggcccgcctggctgaccgcccaacgacccccgcccattgacgtcaataatgacgtatgttcccatagtaacgccaatagggactttccattgacgtcaatgggtggagtatttacggtaaactgcccacttggcagtacatcaagtgtatcatatgccaagtacgccccctattgacgtcaatgacggtaaatggcccgcctggcattatgcccagtacatgaccttatgggactttcctacttggcagtacatctacgtattagtcatcgctattaccatgctgatgcggttttggcagtacatcaatgggcgtggatagcggtttgactcacggggatttccaagtctccaccccattgacgtcaatgggagtttgttttggcaccaaaatcaacgggactttccaaaatgtcgtaacaactccgccccattgacgcaaatgggcggtaggcgtgtacggtgggaggtctatataagcagagctggtttagtgaaccgtcagatcagatctagagatcccgggaccgccaccatgagccccgcggggcccaaggtcccctggttcccaagaaaagtgtcagagctggacaagtgtcatcacctggtcaccaagttcgaccctgacctggacttggaccacccgggcttctcggaccaggtgtaccgccagcgcaggaagctgattgctgagatcgccttccagtacaggcacggcgacccgattccccgtgtggagtacaccgccgaggagattgccacctggaaggaggtctacaccacgctgaagggcctctacgccacgcacgcctgcggggagcacctggaggcctttgctttgctggagcgcttcagcggctaccgggaagacaatatcccccagctggaggacgtctcccgcttcctgaaggagcgcacgggcttccagctgcggcctgtggccggcctgctgtccgcccgggacttcctggccagcctggccttccgcgtgttccagtgcacccagtatatccgccacgcgtcctcgcccatgcactcccctgagccggactgctgccacgagctgctggggcacgtgcccatgctggccgaccgcaccttcgcgcagttctcgcaggacattggcctggcgtccctgggggcctcggatgaggaaattgagaagctgtccacgctgtactggttcacggtggagttcgggctgtgtaagcagaacggggaggtgaaggcctatggtgccgggctgctgtcctcctacggggagctcctgcactgcctgtctgaggagcctgagattcgggccttcgaccctgaggctgcggccgtgcagccctaccaagaccagacgtaccagtcagtctacttcgtgtctgagagcttcagtgacgccaaggacaagctcaggagctatgcctcacgcatccagcgccccttctccgtgaagttcgacccgtacacgctggccatcgacgtgctggacagcccccaggccgtgcggcgctccctggagggtgtccaggatgagctggacacccttgcccatgcgctgagtgccattggctaaagcaggtttccccaactgacacaaaacgtgcaacttgaaactccgcctggtctttccaggtctagaggggtaacactttgtactgcgtttggctccacgctcgatccactggcgagtgttagtaacagcactgttgcttcgtagcggagcatgacggccgtgggaactcctccttggtaacaaggacccacggggccaaaagccacgcccacacgggcccgtcatgtgtgcaaccccagcacggcgactttactgcgaaacccactttaaagtgacattgaaactggtacccacacactggtgacaggctaaggatgcccttcaggtaccccgaggtaacacgcgacactcgggatctgagaaggggactggggcttctataaaagcgctcggtttaaaaagcttctatgcctgaataggtgaccggaggtcggcacctttcctttgcaattactgaccacgccaccatggagaagccgcggggagtcaggtgcaccaatgggttctccgagcgggagctgccgcggcccggggccagcccgcctgccgagaagtcccggccgcccgaggccaagggcgcacagccggccgacgcctggaaggcagggcggcaccgcagcgaggaggaaaaccaggtgaacctccccaaactggcggctgcttactcgtccattctgctctcgctgggcgaggacccccagcggcaggggctgctcaagacgccctggagggcggccaccgccatgcagtacttcaccaagggataccaggagaccatctcagatgtcctgaatgatgctatatttgatgaagatcatgacgagatggtgattgtgaaggacatagatatgttctccatgtgtgagcatcaccttgttccatttgtaggaagggtccatattggctatcttcctaacaagcaagtccttggtctcagtaaacttgccaggattgtagaaatctacagtagacgactacaagttcaagagcgcctcaccaaacagattgcggtggccatcacagaagccttgcagcctgctggcgttggagtagtgattgaagcgacacacatgtgcatggtaatgcgaggcgtgcagaaaatgaacagcaagactgtcactagcaccatgctgggcgtgttccgggaagaccccaagactcgggaggagttcctcacactaatcaggagctgaggccacctaatcaacctctggattacaaaatttgtgaaagattgactggtattcttaactatgttgctccttttacgctatgtggatacgctgctttaatgcctttgtatcatgctattgcttcccgtatggctttcattttctcctccttgtataaatcctggttgctgtctctttatgaggagttgtggcccgttgtcaggcaacgtggcgtggtgtgcactgtgtttgctgacgcaacccccactggttggggcattgccaccacctgtcagctcctttccgggactttcgctttccccctccctattgccacggcggaactcatcgccgcctgccttgcccgctgctggacaggggctcggctgttgggcactgacaattccgtggtgttgtcggggaaatcatcgtcctttcccatatgcagctcacagacatgataagatacattgatgagtttggacaaaccacaactagaatgcagtgaaaaaaatgctttatttgtgaaatttgtgatgctattgctttatttgtaaccattataagctgcaataaacaagttaacaacaacaattgcattcattttatgtttcaggttcagggggaggtgtgggaggttttttaaagcaagtaaaacctctacaaatgtggtattggcccatctctatcggtatcgtagcataaccccttggggcctctaaacgggtcttgaggggttttttgtgcccctcgggccggattgctatctaccggcattggcgcagaaaaaaatgcctgatgcgacgctgcgcgtcttatactcccacatatgccagattcagcaacggatacggcttccccaacttgcccacttccatacgtgtcctccttaccagaaatttatccttaaggtcgtcagctatcctgcaggcgatctctcgatttcgatcaagacattcctttaatggtcttttctggacaccactaggggtcagaagtagttcatcaaactttcttccctccctaatctcattggttaccttgggctatcgaaacttaattaaccagtcaagtcagctacttggcgagatcgacttgtctgggtttcgactacgctcagaattgcgtcagtcaagttcgatctggtccttgctattgcacccgttctccgattacgagtttcatttaaatcatgtgagcaaaaggccagcaaaaggccaggaaccgtaaaaaggccgcgttgctggcgtttttccataggctccgcccccctgacgagcatcacaaaaatcgacgctcaagtcagaggtggcgaaacccgacaggactataaagataccaggcgtttccccctggaagctccctcgtgcgctctcctgttccgaccctgccgcttaccggatacctgtccgcctttctcccttcgggaagcgtggcgctttctcatagctcacgctgtaggtatctcagttcggtgtaggtcgttcgctccaagctgggctgtgtgcacgaaccccccgttcagcccgaccgctgcgccttatccggtaactatcgtcttgagtccaacccggtaagacacgacttatcgccactggcagcagccactggtaacaggattagcagagcgaggtatgtaggcggtgctacagagttcttgaagtggtggcctaactacggctacactagaagaacagtatttggtatctgcgctctgctgaagccagttaccttcggaaaaagagttggtagctcttgatccggcaaacaaaccaccgctggtagcggtggtttttttgtttgcaagcagcagattacgcgcagaaaaaaaggatctcaagaagatcctttgatcttttctacggggtctgacgctcagtggaacgaaaactcacgttaagggattttggtcatgagattatcaaaaaggatcttcacctagatccttttaaattaaaaatgaagttttaaatcaatctaaagtatatatgagtaaacttggtctgacagttaccaatgcttaatcagtgaggcacctatctcagcgatctgtctatttcgttcatccatagttgcatttaaatttccgaactctccaaggccctcgtcggaaaatcttcaaacctttcgtccgatccatcttgcaggctacctctcgaacgaactatcgcaagtctcttggccggccttgcgccttggctattgcttggcagcgcctatcgccaggtattactccaatcccgaatatccgagatcgggatcacccgagagaagttcaacctacatcctcaatcccgatctatccgagatccgaggaatatcgaaatcggggcgcgcctggtgtaccgagaacgatcctctcagtgcgagtctcgacgatccatatcgttgcttggcagtcagccagtcggaatccagcttgggacccaggaagtccaatcgtcagatattgtactcaagcctggtcacggcagcgtaccgatctgtttaaacctagatattgatagtctgatcggtcaacgtataatcgagtcctagcttttgcaaacatctatcaagagacaggatcagcaggaggctttcgcatgagtattcaacatttccgtgtcgcccttattcccttttttgcggcattttgccttcctgtttttgctcacccagaaacgctggtgaaagtaaaagatgctgaagatcagttgggtgcgcgagtgggttacatcgaactggatctcaacagcggtaagatccttgagagttttcgccccgaagaacgctttccaatgatgagcacttttaaagttctgctatgtggcgcggtattatcccgtattgacgccgggcaagagcaactcggtcgccgcatacactattctcagaatgacttggttgagtattcaccagtcacagaaaagcatcttacggatggcatgacagtaagagaattatgcagtgctgccataaccatgagtgataacactgcggccaacttacttctgacaacgattggaggaccgaaggagctaaccgcttttttgcacaacatgggggatcatgtaactcgccttgatcgttgggaaccggagctgaatgaagccataccaaacgacgagcgtgacaccacgatgcctgtagcaatggcaacaaccttgcgtaaactattaactggcgaactacttactctagcttcccggcaacagttgatagactggatggaggcggataaagttgcaggaccacttctgcgctcggcccttccggctggctggtttattgctgataaatctggagccggtgagcgtgggtctcgcggtatcattgcagcactggggccagatggtaagccctcccgtatcgtagttatctacacgacggggagtcaggcaactatggatgaacgaaatagacagatcgctgagataggtgcctcactgattaagcattggtaaccgattctaggtgcattggcgcagaaaaaaatgcctgatgcgacgctgcgcgtcttatactcccacatatgccagattcagcaacggatacggcttccccaacttgcccacttccatacgtgtcctccttaccagaaatttatccttaagatcccgaatcgtttaaactcgactctggctctatcgaatctccgtcgtttcgagcttacgcgaacagccgtggcgctcatttgctcgtcgggcatcgaatctcgtcagctatcgtcagcttacctttttggca

SEQ ID NO: 19 - DNA, 6390 bp, Unknown
  The genetic construct as shown in Fig. 11. This embodiment includes a CMV promoter and murine GCH1.
ggcgatcgcggctcccgacatcttggaccattagctccacaggtatcttcttccctctagtggtcataacagcagcttcagctacctctcaattcaaaaaacccctcaagacccgtttagaggccccaaggggttatgctatcaatcgttgcgttacacacacaaaaaaccaacacacatccatcttcgatggatagcgattttattatctaactgctgatcgagtgtagccagatctagtaatcaattacggggtcattagttcatagcccatatatggagttccgcgttacataacttacggtaaatggcccgcctggctgaccgcccaacgacccccgcccattgacgtcaataatgacgtatgttcccatagtaacgccaatagggactttccattgacgtcaatgggtggagtatttacggtaaactgcccacttggcagtacatcaagtgtatcatatgccaagtacgccccctattgacgtcaatgacggtaaatggcccgcctggcattatgcccagtacatgaccttatgggactttcctacttggcagtacatctacgtattagtcatcgctattaccatgctgatgcggttttggcagtacatcaatgggcgtggatagcggtttgactcacggggatttccaagtctccaccccattgacgtcaatgggagtttgttttggcaccaaaatcaacgggactttccaaaatgtcgtaacaactccgccccattgacgcaaatgggcggtaggcgtgtacggtgggaggtctatataagcagagctggtttagtgaaccgtcagatcagatctagagatcccgggaccgccaccatgagccccgcggggcccaaggtcccctggttcccaagaaaagtgtcagagctggacaagtgtcatcacctggtcaccaagttcgaccctgacctggacttggaccacccgggcttctcggaccaggtgtaccgccagcgcaggaagctgattgctgagatcgccttccagtacaggcacggcgacccgattccccgtgtggagtacaccgccgaggagattgccacctggaaggaggtctacaccacgctgaagggcctctacgccacgcacgcctgcggggagcacctggaggcctttgctttgctggagcgcttcagcggctaccgggaagacaatatcccccagctggaggacgtctcccgcttcctgaaggagcgcacgggcttccagctgcggcctgtggccggcctgctgtccgcccgggacttcctggccagcctggccttccgcgtgttccagtgcacccagtatatccgccacgcgtcctcgcccatgcactcccctgagccggactgctgccacgagctgctggggcacgtgcccatgctggccgaccgcaccttcgcgcagttctcgcaggacattggcctggcgtccctgggggcctcggatgaggaaattgagaagctgtccacgctgtactggttcacggtggagttcgggctgtgtaagcagaacggggaggtgaaggcctatggtgccgggctgctgtcctcctacggggagctcctgcactgcctgtctgaggagcctgagattcgggccttcgaccctgaggctgcggccgtgcagccctaccaagaccagacgtaccagtcagtctacttcgtgtctgagagcttcagtgacgccaaggacaagctcaggagctatgcctcacgcatccagcgccccttctccgtgaagttcgacccgtacacgctggccatcgacgtgctggacagcccccaggccgtgcggcgctccctggagggtgtccaggatgagctggacacccttgcccatgcgctgagtgccattggctaacgcgcgaaacgcgcgccggtgaaacagaccctgaactttgatctgctgaaactggcgggcgatgtggaaagcaacccgggcccgatggagaagccgcggggagtcaggtgcaccaatgggttctccgagcgggagctgccgcggcccggggccagcccgcctgccgagaagtcccggccgcccgaggccaagggcgcacagccggccgacgcctggaaggcagggcggcaccgcagcgaggaggaaaaccaggtgaacctccccaaactggcggctgcttactcgtccattctgctctcgctgggcgaggacccccagcggcaggggctgctcaagacgccctggagggcggccaccgccatgcagtacttcaccaagggataccaggagaccatctcagatgtcctgaatgatgctatatttgatgaagatcatgacgagatggtgattgtgaaggacatagatatgttctccatgtgtgagcatcaccttgttccatttgtaggaagggtccatattggctatcttcctaacaagcaagtccttggtctcagtaaacttgccaggattgtagaaatctacagtagacgactacaagttcaagagcgcctcaccaaacagattgcggtggccatcacagaagccttgcagcctgctggcgttggagtagtgattgaagcgacacacatgtgcatggtaatgcgaggcgtgcagaaaatgaacagcaagactgtcactagcaccatgctgggcgtgttccgggaagaccccaagactcgggaggagttcctcacactaatcaggagctgaggccacctaatcaacctctggattacaaaatttgtgaaagattgactggtattcttaactatgttgctccttttacgctatgtggatacgctgctttaatgcctttgtatcatgctattgcttcccgtatggctttcattttctcctccttgtataaatcctggttgctgtctctttatgaggagttgtggcccgttgtcaggcaacgtggcgtggtgtgcactgtgtttgctgacgcaacccccactggttggggcattgccaccacctgtcagctcctttccgggactttcgctttccccctccctattgccacggcggaactcatcgccgcctgccttgcccgctgctggacaggggctcggctgttgggcactgacaattccgtggtgttgtcggggaaatcatcgtcctttcccatatgcagctcacagacatgataagatacattgatgagtttggacaaaccacaactagaatgcagtgaaaaaaatgctttatttgtgaaatttgtgatgctattgctttatttgtaaccattataagctgcaataaacaagttaacaacaacaattgcattcattttatgtttcaggttcagggggaggtgtgggaggttttttaaagcaagtaaaacctctacaaatgtggtattggcccatctctatcggtatcgtagcataaccccttggggcctctaaacgggtcttgaggggttttttgtgcccctcgggccggattgctatctaccggcattggcgcagaaaaaaatgcctgatgcgacgctgcgcgtcttatactcccacatatgccagattcagcaacggatacggcttccccaacttgcccacttccatacgtgtcctccttaccagaaatttatccttaaggtcgtcagctatcctgcaggcgatctctcgatttcgatcaagacattcctttaatggtcttttctggacaccactaggggtcagaagtagttcatcaaactttcttccctccctaatctcattggttaccttgggctatcgaaacttaattaaccagtcaagtcagctacttggcgagatcgacttgtctgggtttcgactacgctcagaattgcgtcagtcaagttcgatctggtccttgctattgcacccgttctccgattacgagtttcatttaaatcatgtgagcaaaaggccagcaaaaggccaggaaccgtaaaaaggccgcgttgctggcgtttttccataggctccgcccccctgacgagcatcacaaaaatcgacgctcaagtcagaggtggcgaaacccgacaggactataaagataccaggcgtttccccctggaagctccctcgtgcgctctcctgttccgaccctgccgcttaccggatacctgtccgcctttctcccttcgggaagcgtggcgctttctcatagctcacgctgtaggtatctcagttcggtgtaggtcgttcgctccaagctgggctgtgtgcacgaaccccccgttcagcccgaccgctgcgccttatccggtaactatcgtcttgagtccaacccggtaagacacgacttatcgccactggcagcagccactggtaacaggattagcagagcgaggtatgtaggcggtgctacagagttcttgaagtggtggcctaactacggctacactagaagaacagtatttggtatctgcgctctgctgaagccagttaccttcggaaaaagagttggtagctcttgatccggcaaacaaaccaccgctggtagcggtggtttttttgtttgcaagcagcagattacgcgcagaaaaaaaggatctcaagaagatcctttgatcttttctacggggtctgacgctcagtggaacgaaaactcacgttaagggattttggtcatgagattatcaaaaaggatcttcacctagatccttttaaattaaaaatgaagttttaaatcaatctaaagtatatatgagtaaacttggtctgacagttaccaatgcttaatcagtgaggcacctatctcagcgatctgtctatttcgttcatccatagttgcatttaaatttccgaactctccaaggccctcgtcggaaaatcttcaaacctttcgtccgatccatcttgcaggctacctctcgaacgaactatcgcaagtctcttggccggccttgcgccttggctattgcttggcagcgcctatcgccaggtattactccaatcccgaatatccgagatcgggatcacccgagagaagttcaacctacatcctcaatcccgatctatccgagatccgaggaatatcgaaatcggggcgcgcctggtgtaccgagaacgatcctctcagtgcgagtctcgacgatccatatcgttgcttggcagtcagccagtcggaatccagcttgggacccaggaagtccaatcgtcagatattgtactcaagcctggtcacggcagcgtaccgatctgtttaaacctagatattgatagtctgatcggtcaacgtataatcgagtcctagcttttgcaaacatctatcaagagacaggatcagcaggaggctttcgcatgagtattcaacatttccgtgtcgcccttattcccttttttgcggcattttgccttcctgtttttgctcacccagaaacgctggtgaaagtaaaagatgctgaagatcagttgggtgcgcgagtgggttacatcgaactggatctcaacagcggtaagatccttgagagttttcgccccgaagaacgctttccaatgatgagcacttttaaagttctgctatgtggcgcggtattatcccgtattgacgccgggcaagagcaactcggtcgccgcatacactattctcagaatgacttggttgagtattcaccagtcacagaaaagcatcttacggatggcatgacagtaagagaattatgcagtgctgccataaccatgagtgataacactgcggccaacttacttctgacaacgattggaggaccgaaggagctaaccgcttttttgcacaacatgggggatcatgtaactcgccttgatcgttgggaaccggagctgaatgaagccataccaaacgacgagcgtgacaccacgatgcctgtagcaatggcaacaaccttgcgtaaactattaactggcgaactacttactctagcttcccggcaacagttgatagactggatggaggcggataaagttgcaggaccacttctgcgctcggcccttccggctggctggtttattgctgataaatctggagccggtgagcgtgggtctcgcggtatcattgcagcactggggccagatggtaagccctcccgtatcgtagttatctacacgacggggagtcaggcaactatggatgaacgaaatagacagatcgctgagataggtgcctcactgattaagcattggtaaccgattctaggtgcattggcgcagaaaaaaatgcctgatgcgacgctgcgcgtcttatactcccacatatgccagattcagcaacggatacggcttccccaacttgcccacttccatacgtgtcctccttaccagaaatttatccttaagatcccgaatcgtttaaactcgactctggctctatcgaatctccgtcgtttcgagcttacgcgaacagccgtggcgctcatttgctcgtcgggcatcgaatctcgtcagctatcgtcagcttacctttttggca

SEQ ID NO: 20 - DNA, 6380 bp, Unknown
  The genetic construct is shown in Fig. 12. This embodiment includes a CMV promoter and murine GCH1.
ggcgatcgcggctcccgacatcttggaccattagctccacaggtatcttcttccctctagtggtcataacagcagcttcagctacctctcaattcaaaaaacccctcaagacccgtttagaggccccaaggggttatgctatcaatcgttgcgttacacacacaaaaaaccaacacacatccatcttcgatggatagcgattttattatctaactgctgatcgagtgtagccagatctagtaatcaattacggggtcattagttcatagcccatatatggagttccgcgttacataacttacggtaaatggcccgcctggctgaccgcccaacgacccccgcccattgacgtcaataatgacgtatgttcccatagtaacgccaatagggactttccattgacgtcaatgggtggagtatttacggtaaactgcccacttggcagtacatcaagtgtatcatatgccaagtacgccccctattgacgtcaatgacggtaaatggcccgcctggcattatgcccagtacatgaccttatgggactttcctacttggcagtacatctacgtattagtcatcgctattaccatgctgatgcggttttggcagtacatcaatgggcgtggatagcggtttgactcacggggatttccaagtctccaccccattgacgtcaatgggagtttgttttggcaccaaaatcaacgggactttccaaaatgtcgtaacaactccgccccattgacgcaaatgggcggtaggcgtgtacggtgggaggtctatataagcagagctggtttagtgaaccgtcagatcagatctagagatcccgggaccgccaccatgagccccgcggggcccaaggtcccctggttcccaagaaaagtgtcagagctggacaagtgtcatcacctggtcaccaagttcgaccctgacctggacttggaccacccgggcttctcggaccaggtgtaccgccagcgcaggaagctgattgctgagatcgccttccagtacaggcacggcgacccgattccccgtgtggagtacaccgccgaggagattgccacctggaaggaggtctacaccacgctgaagggcctctacgccacgcacgcctgcggggagcacctggaggcctttgctttgctggagcgcttcagcggctaccgggaagacaatatcccccagctggaggacgtctcccgcttcctgaaggagcgcacgggcttccagctgcggcctgtggccggcctgctgtccgcccgggacttcctggccagcctggccttccgcgtgttccagtgcacccagtatatccgccacgcgtcctcgcccatgcactcccctgagccggactgctgccacgagctgctggggcacgtgcccatgctggccgaccgcaccttcgcgcagttctcgcaggacattggcctggcgtccctgggggcctcggatgaggaaattgagaagctgtccacgctgtactggttcacggtggagttcgggctgtgtaagcagaacggggaggtgaaggcctatggtgccgggctgctgtcctcctacggggagctcctgcactgcctgtctgaggagcctgagattcgggccttcgaccctgaggctgcggccgtgcagccctaccaagaccagacgtaccagtcagtctacttcgtgtctgagagcttcagtgacgccaaggacaagctcaggagctatgcctcacgcatccagcgccccttctccgtgaagttcgacccgtacacgctggccatcgacgtgctggacagcccccaggccgtgcggcgctccctggagggtgtccaggatgagctggacacccttgcccatgcgctgagtgccattggcggaggtggcgggtccgggggcgggggtagcggtggcgggggctccgccaccatggagaagggccctgtgcgggcaccggcggagaagccgcggggcgccaggtgcagcaatgggttccccgagcgggatccgccgcggcccgggcccagcaggccggcggagaagcccccgcggcccgaggccaagagcgcgcagcccgcggacggctggaagggcgagcggccccgcagcgaggaggataacgagctgaacctccctaacctggcagccgcctactcgtccatcctgagctcgctgggcgagaacccccagcggcaagggctgctcaagacgccctggagggcggcctcggccatgcagttcttcaccaagggctaccaggagaccatctcagatgtcctaaacgatgctatatttgatgaagatcatgatgagatggtgattgtgaaggacatagacatgttttccatgtgtgagcatcacttggttccatttgttggaaaggtccatattggttatcttcctaacaagcaagtccttggcctcagcaaacttgcgaggattgtagaaatctatagtagaagactacaagttcaggagcgccttacaaaacaaattgctgtagcaatcacggaagccttgcggcctgctggagtcggggtagtggttgaagcaacacacatgtgtatggtaatgcgaggtgtacagaaaatgaacagcaaaactgtgaccagcacaatgttgggtgtgttccgggaggatccaaagactcgggaagagttcctgactctcattaggagctgagccacctaatcaacctctggattacaaaatttgtgaaagattgactggtattcttaactatgttgctccttttacgctatgtggatacgctgctttaatgcctttgtatcatgctattgcttcccgtatggctttcattttctcctccttgtataaatcctggttgctgtctctttatgaggagttgtggcccgttgtcaggcaacgtggcgtggtgtgcactgtgtttgctgacgcaacccccactggttggggcattgccaccacctgtcagctcctttccgggactttcgctttccccctccctattgccacggcggaactcatcgccgcctgccttgcccgctgctggacaggggctcggctgttgggcactgacaattccgtggtgttgtcggggaaatcatcgtcctttcccatatgcagctcacagacatgataagatacattgatgagtttggacaaaccacaactagaatgcagtgaaaaaaatgctttatttgtgaaatttgtgatgctattgctttatttgtaaccattataagctgcaataaacaagttaacaacaacaattgcattcattttatgtttcaggttcagggggaggtgtgggaggttttttaaagcaagtaaaacctctacaaatgtggtattggcccatctctatcggtatcgtagcataaccccttggggcctctaaacgggtcttgaggggttttttgtgcccctcgggccggattgctatctaccggcattggcgcagaaaaaaatgcctgatgcgacgctgcgcgtcttatactcccacatatgccagattcagcaacggatacggcttccccaacttgcccacttccatacgtgtcctccttaccagaaatttatccttaaggtcgtcagctatcctgcaggcgatctctcgatttcgatcaagacattcctttaatggtcttttctggacaccactaggggtcagaagtagttcatcaaactttcttccctccctaatctcattggttaccttgggctatcgaaacttaattaaccagtcaagtcagctacttggcgagatcgacttgtctgggtttcgactacgctcagaattgcgtcagtcaagttcgatctggtccttgctattgcacccgttctccgattacgagtttcatttaaatcatgtgagcaaaaggccagcaaaaggccaggaaccgtaaaaaggccgcgttgctggcgtttttccataggctccgcccccctgacgagcatcacaaaaatcgacgctcaagtcagaggtggcgaaacccgacaggactataaagataccaggcgtttccccctggaagctccctcgtgcgctctcctgttccgaccctgccgcttaccggatacctgtccgcctttctcccttcgggaagcgtggcgctttctcatagctcacgctgtaggtatctcagttcggtgtaggtcgttcgctccaagctgggctgtgtgcacgaaccccccgttcagcccgaccgctgcgccttatccggtaactatcgtcttgagtccaacccggtaagacacgacttatcgccactggcagcagccactggtaacaggattagcagagcgaggtatgtaggcggtgctacagagttcttgaagtggtggcctaactacggctacactagaagaacagtatttggtatctgcgctctgctgaagccagttaccttcggaaaaagagttggtagctcttgatccggcaaacaaaccaccgctggtagcggtggtttttttgtttgcaagcagcagattacgcgcagaaaaaaaggatctcaagaagatcctttgatcttttctacggggtctgacgctcagtggaacgaaaactcacgttaagggattttggtcatgagattatcaaaaaggatcttcacctagatccttttaaattaaaaatgaagttttaaatcaatctaaagtatatatgagtaaacttggtctgacagttaccaatgcttaatcagtgaggcacctatctcagcgatctgtctatttcgttcatccatagttgcatttaaatttccgaactctccaaggccctcgtcggaaaatcttcaaacctttcgtccgatccatcttgcaggctacctctcgaacgaactatcgcaagtctcttggccggccttgcgccttggctattgcttggcagcgcctatcgccaggtattactccaatcccgaatatccgagatcgggatcacccgagagaagttcaacctacatcctcaatcccgatctatccgagatccgaggaatatcgaaatcggggcgcgcctggtgtaccgagaacgatcctctcagtgcgagtctcgacgatccatatcgttgcttggcagtcagccagtcggaatccagcttgggacccaggaagtccaatcgtcagatattgtactcaagcctggtcacggcagcgtaccgatctgtttaaacctagatattgatagtctgatcggtcaacgtataatcgagtcctagcttttgcaaacatctatcaagagacaggatcagcaggaggctttcgcatgagtattcaacatttccgtgtcgcccttattcccttttttgcggcattttgccttcctgtttttgctcacccagaaacgctggtgaaagtaaaagatgctgaagatcagttgggtgcgcgagtgggttacatcgaactggatctcaacagcggtaagatccttgagagttttcgccccgaagaacgctttccaatgatgagcacttttaaagttctgctatgtggcgcggtattatcccgtattgacgccgggcaagagcaactcggtcgccgcatacactattctcagaatgacttggttgagtattcaccagtcacagaaaagcatcttacggatggcatgacagtaagagaattatgcagtgctgccataaccatgagtgataacactgcggccaacttacttctgacaacgattggaggaccgaaggagctaaccgcttttttgcacaacatgggggatcatgtaactcgccttgatcgttgggaaccggagctgaatgaagccataccaaacgacgagcgtgacaccacgatgcctgtagcaatggcaacaaccttgcgtaaactattaactggcgaactacttactctagcttcccggcaacagttgatagactggatggaggcggataaagttgcaggaccacttctgcgctcggcccttccggctggctggtttattgctgataaatctggagccggtgagcgtgggtctcgcggtatcattgcagcactggggccagatggtaagccctcccgtatcgtagttatctacacgacggggagtcaggcaactatggatgaacgaaatagacagatcgctgagataggtgcctcactgattaagcattggtaaccgattctaggtgcattggcgcagaaaaaaatgcctgatgcgacgctgcgcgtcttatactcccacatatgccagattcagcaacggatacggcttccccaacttgcccacttccatacgtgtcctccttaccagaaatttatccttaagatcccgaatcgtttaaactcgactctggctctatcgaatctccgtcgtttcgagcttacgcgaacagccgtggcgctcatttgctcgtcgggcatcgaatctcgtcagctatcgtcagcttacctttttggca

SEQ ID NO: 21 - protein, 497 aa, Homo sapiens
MPTPDATTPQAKGFRRAVSELDAKQAEAIMSPRFIGRRQSLIEDARKEREAAVAAAAAAVPSEPGDPLEAVAFEEKEGKAVLNLLFSPRATKPSALSRAVKVFETFEAKIHHLETRPAQRPRAGGPHLEYFVRLEVRRGDLAALLSGVRQVSEDVRSPAGPKVPWFPRKVSELDKCHHLVTKFDPDLDLDHPGFSDQVYRQRRKLIAEIAFQYRHGDPIPRVEYTAEEIATWKEVYTTLKGLYATHACGEHLEAFALLERFSGYREDNIPQLEDVSRFLKERTGFQLRPVAGLLSARDFLASLAFRVFQCTQYIRHASSPMHSPEPDCCHELLGHVPMLADRTFAQFSQDIGLASLGASDEEIEKLSTLYWFTVEFGLCKQNGEVKAYGAGLLSSYGELLHCLSEEPEIRAFDPEAAAVQPYQDQTYQSVYFVSESFSDAKDKLRSYASRIQRPFSVKFDPYTLAIDVLDSPQAVRRSLEGVQDELDTLAHALSAIG

SEQ ID NO: 22 - protein, 342 aa, Homo sapiens
MSPAGPKVPWFPRKVSELDKCHHLVTKFDPDLDLDHPGFSDQVYRQRRKLIAEIAFQYRHGDPIPRVEYTAEEIATWKEVYTTLKGLYATHACGEHLEAFALLERFSGYREDNIPQLEDVSRFLKERTGFQLRPVAGLLSARDFLASLAFRVFQCTQYIRHASSPMHSPEPDCCHELLGHVPMLADRTFAQFSQDIGLASLGASDEEIEKLSTLYWFTVEFGLCKQNGEVKAYGAGLLSSYGELLHCLSEEPEIRAFDPEAAAVQPYQDQTYQSVYFVSESFSDAKDKLRSYASRIQRPFSVKFDPYTLAIDVLDSPQAVRRSLEGVQDELDTLAHALSAIG

SEQ ID NO: 23 - protein, 250 aa, Homo sapiens
MEKGPVRAPAEKPRGARCSNGFPERDPPRPGPSRPAEKPPRPEAKSAQPADGWKGERPRSEEDNELNLPNLAAAYSSILSSLGENPQRQGLLKTPWRAASAMQFFTKGYQETISDVLNDAIFDEDHDEMVIVKDIDMFSMCEHHLVPFVGKVHIGYLPNKQVLGLSKLARIVEIYSRRLQVQERLTKQIAVAITEALRPAGVGVVVEATHMCMVMRGVQKMNSKTVTSTMLGVFREDPKTREEFLTLIRS

SEQ ID NO: 24 - protein, 15 aa, Unknown
  Flexible linker sequence.
GGGGSGGGGSGGGGS

SEQ ID NO: 25 - DNA, 663 bp, Unknown
  CMV promoter
acgcgtggagctagttattaatagtaatcaattacggggtcattagttcatagcccatatatggagttccgcgttacataacttacggtaaatggcccgcctggctgaccgcccaacgacccccgcccattgacgtcaataatgacgtatgttcccatagtaacgtcaatagggactttccattgacgtcaatgggtggagtatttacggtaaactgcccacttggcagtacatcaagtgtatcatatgccaagtacgccccctattgacgtcaatgacggtaaatggcccgcctggcattatgcccagtacatgaccttatgggactttcctacttggcagtacatctacgtattagtcatcgctattaccatggtgatgcggttttggcagtacatcaatgggcgtggatagcggtttgactcacggggatttccaagtctccaccccattgacgtcaatgggagtttgttttgcaccaaaatcaacgggactttccaaaatgtcgtaacaactccgccccattgacgcaaatgggcggtaggcgtgtacggtgggaggtctatataagcagagctcgtttagtgaaccgtcagatcgcctggagacgccatccacgctgttttgacctccatagaagacaccgggaccgatccagcctcc

SEQ ID NO: 26 - DNA, 1338 bp, Unknown
  OIPR sequence
attgggatcttcacacagcaggtaaggttgcgggccgggcctgggccgggtccgggccgggtattgcccgcctaatgagcgggcttttttttcttaccccttcttccgcttcctcgctcactgactcgctgcgctcggtcgttcggctgcggcgagcggtatcagctcactcaaaggcggtaatacggttatccacagaatcaggggataacgcaggaaagaacatgtgagcaaaaggccagcaaaaggccaggaaccgtaaaaaggccgcgttgctggcgtttttccataggctccgcccccctgacgagcatcacaaaaatcgacgctcaagtcagaggtggcgaaacccgacaggactataaagataccaggcgtttccccctggaagctccctcgtgcgctctcctgttccgaccctgccgcttaccggatacctgtccgcctttctcccttcgggaagcgtggcgctttctcatagctcacgctgtaggtatctcagttcggtgtaggtcgttcgctccaagctgggctgtgtgcacgaaccccccgttcagcccgaccgctgcgccttatccggtaactatcgtcttgagtccaacccggtaagacacgacttatcgccactggcagcagccactggtaacaggattagcagagcgaggtatgtaggcggtgctacagagttcttgaagtggtggcctaactacggctacactagaagaacagtatttggtatctgcgctctgctgaagccagttaccttcggaaaaagagttggtagctcttgatccggcaaacaaaccaccgctggtagcggtggtttttttgtttgcaagcagcagattacgcgcagaaaaaaaggatctcaagaagatcctttgatcttttctacggggtctgacgctcagtggaacgaaaactcacgttaagggattttggtcatgagattatcaaaaaggatcttcacctagatccttttaaattaaaaatgaagttttaaatcaatctaaagtatatatgagtaaacttggtctgacagttaccaatgcttaatcagtgaggcacctatctcagcgatctgtctatttcgttcatccatagttgcctgactcctgcaaaccacgttgtggtagaattggtaaagagagtcgtgtaaaatatcgagttcgcacatcttgttgtctgattattgatttttggcgaaaccatttgatcatatgacaagatgtgtatctaccttaacttaatgattttgataaaaatcattaggtaccccggcccgcactgacccctggtgttgctttttttttttaggccgcaagctgaagcgtgtcc

SEQ ID NO: 27 - DNA, 60 bp, Unknown
  E2A sequence
cagtgtactaattatgctctcttgaaattggctggagatgttgagagcaaccctggacct

SEQ ID NO: 28 - DNA, 66 bp, Unknown
  F2A sequence.
gtgaaacagactttgaattttgaccttctcaagttggcgggagacgtggagtccaaccctggacct

SEQ ID NO: 29 - DNA, 57 bp, Unknown
  P2A sequence.
gccacgaacttctctctgttaaagcaagcaggagatgttgaagaaaaccccgggcct

SEQ ID NO: 30 - DNA, 54 bp, Unknown
  T2A sequence.
gagggcaggggaagtcttctaacatgcggggacgtggaggaaaatcccggcccc

SEQ ID NO: 31 - DNA, 9 bp, Unknown
  glycine-serine-glycine spacer sequence.
ggaagcgga